European Patent Specification EP 3 310 812 B1, published July 30, 2025. Title: ANTI-HER2 ANTIBODIES AND METHODS OF USE. Applicant: GENENTECH, INC. ET AL. The sequence listing filed with the application follows.

SEQUENCE LISTING (89 sequences)

SEQ ID NO: 1 - protein, 107 aa, Artificial Sequence [sequence omitted]

SEQ ID NO: 2 - protein, 120 aa, Artificial Sequence [sequence omitted]

SEQ ID NO: 3 - protein, 107 aa, Artificial Sequence [sequence omitted]

SEQ ID NO: 4 - protein, 120 aa, Artificial Sequence [sequence omitted]

SEQ ID NO: 5 - protein, 120 aa, Artificial Sequence
  source: /note="Description of Artificial Sequence: Synthetic polypeptide"
  MOD_RES (56)..(56): Any amino acid except Gly
EVQLVESGGGLVQPGGSLRLSCAASGFNIKDTYIHWVRQAPGKGLEWVARIYPTNXYTRYADSVKGRFTISADTSKNTAYLQMNSLRAEDTAVYYCSRWGGDGFYAMDYWGQGTLVTVSS

SEQ ID NO: 6 - protein, 107 aa, Artificial Sequence
  source: /note="Description of Artificial Sequence: Synthetic polypeptide"
DIQMTQSPSSLSASVGDRVTITCRASQDVDTAVAWYQQKPGKAPKLLIYSASFLYSGVPSRFSGSRSGTDFTLTISSLQPEDFATYYCQQHYTTPPTFGQGTKVEIK

SEQ ID NO: 7 - protein, 120 aa, Artificial Sequence
  source: /note="Description of Artificial Sequence: Synthetic polypeptide"
EVQLVESGGGLVQPGGSLRLSCAASGFNIKDTYIHWVRQAPGKGLEWVARIYPTEGYTRYADSVKGRFTISADTSKNTAYLQMNSLRAEDTAVYYCSRWGGDSFYAMDYWGQGTLVTVSS

SEQ ID NO: 8 - protein, 107 aa, Artificial Sequence
  source: /note="Description of Artificial Sequence: Synthetic polypeptide"
DIQMTQSPSSLSASVGDRVTITCRASQDVSTAVAWYQQKPGKAPKLLIYSASFLYSGVPSRFSGSRSGTDFTLTISSLQPEDFATYYCQQHYTTPPTFGQGTKVEIK

SEQ ID NO: 9 - protein, 120 aa, Artificial Sequence
  source: /note="Description of Artificial Sequence: Synthetic polypeptide"
EVQLVESGGGLVQPGGSLRLSCAASGFNIKDTYIHWVRQAPGKGLEWVARIYPTEGYTRYADSVKGRFTISADTSKNTAYLQMNSLRAEDTAVYYCSRWGGTGFYAMDYWGQGTLVTVSS

SEQ ID NO: 10 - protein, 107 aa, Artificial Sequence; identical to SEQ ID NO: 8
  source: /note="Description of Artificial Sequence: Synthetic polypeptide"

SEQ ID NO: 11 - protein, 120 aa, Artificial Sequence
  source: /note="Description of Artificial Sequence: Synthetic polypeptide"
EVQLVESGGGLVQPGGSLRLSCAASGFNIKDTYIHWVRQAPGKGLEWVARIYPTNAYTRYADSVKGRFTISADTSKNTAYLQMNSLRAEDTAVYYCSRWGGTGFYAMDYWGQGTLVTVSS

SEQ ID NO: 12 - protein, 107 aa, Artificial Sequence; identical to SEQ ID NO: 8
  source: /note="Description of Artificial Sequence: Synthetic polypeptide"

SEQ ID NO: 13 - protein, 120 aa, Artificial Sequence
  source: /note="Description of Artificial Sequence: Synthetic polypeptide"
EVQLVESGGGLVQPGGSLRLSCAASGFNIKDTYIHWVRQAPGKGLEWVARIYPTNGYTRYADSVKGRFTISADTSKNTAYLQMNSLRAEDTAVYYCSRWGGDSFYAMDYWGQGTLVTVSS

SEQ ID NO: 14 - protein, 107 aa, Artificial Sequence
  source: /note="Description of Artificial Sequence: Synthetic polypeptide"
DIQMTQSPSSLSASVGDRVTITCRASQDVTTAVAWYQQKPGKAPKLLIYSASFLYSGVPSRFSGSRSGTDFTLTISSLQPEDFATYYCQQHYTTPPTFGQGTKVEIK

SEQ ID NO: 15 - protein, 120 aa, Artificial Sequence; identical to SEQ ID NO: 11
  source: /note="Description of Artificial Sequence: Synthetic polypeptide"

SEQ ID NO: 16 - protein, 107 aa, Artificial Sequence; identical to SEQ ID NO: 8
  source: /note="Description of Artificial Sequence: Synthetic polypeptide"

SEQ ID NO: 17 - protein, 120 aa, Artificial Sequence
  source: /note="Description of Artificial Sequence: Synthetic polypeptide"
EVQLVESGGGLVQPGGSLRLSCAASGFNIKDTYIHWVRQAPGKGLEWVARIYPTNGYTRYADSVKGRFTISADTSKNTAYLQMNSLRAEDTAVYYCSRWGGTGFYAMDYWGQGTLVTVSS

SEQ ID NO: 18 - protein, 107 aa, Artificial Sequence; identical to SEQ ID NO: 8
  source: /note="Description of Artificial Sequence: Synthetic polypeptide"

SEQ ID NO: 19 - protein, 120 aa, Artificial Sequence
  source: /note="Description of Artificial Sequence: Synthetic polypeptide"
EVQLVESGGGLVQPGGSLRLSCAASGFNIKDTYIHWVRQAPGKGLEWVARIYPTNGYTRYADSVKGRFTISADTSKNTAYLQMNSLRAEDTAVYYCSRWGGEGFYAMDYWGQGTLVTVSS

SEQ ID NO: 20 - protein, 107 aa, Artificial Sequence; identical to SEQ ID NO: 6
  source: /note="Description of Artificial Sequence: Synthetic polypeptide"

SEQ ID NO: 21 - protein, 120 aa, Artificial Sequence; identical to SEQ ID NO: 11
  source: /note="Description of Artificial Sequence: Synthetic polypeptide"

SEQ ID NO: 22 - protein, 107 aa, Artificial Sequence; identical to SEQ ID NO: 14
  source: /note="Description of Artificial Sequence: Synthetic polypeptide"

SEQ ID NO: 23 - protein, 120 aa, Artificial Sequence; identical to SEQ ID NO: 17
  source: /note="Description of Artificial Sequence: Synthetic polypeptide"

SEQ ID NO: 24 - protein, 107 aa, Artificial Sequence; identical to SEQ ID NO: 8
  source: /note="Description of Artificial Sequence: Synthetic polypeptide"

SEQ ID NO: 25 - protein, 120 aa, Artificial Sequence
  source: /note="Description of Artificial Sequence: Synthetic polypeptide"
EVQLVESGGGLVQPGGSLRLSCAASGFNIKDTYIHWVRQAPGKGLEWVARIYPTNAYTRYADSVKGRFTISADTSKNTAYLQMNSLRAEDTAVYYCSRWGGDSFYAMDYWGQGTLVTVSS

SEQ ID NO: 26 - protein, 120 aa, Artificial Sequence
  source: /note="Description of Artificial Sequence: Synthetic polypeptide"
EVQLVESGGGLVQPGGSLRLSCAASGFNIKDTYIHWVRQAPGKGLEWVARIYPTNAYTRYADSVKGRFTISADTSKNTAYLQMNSLRAEDTAVYYCSRWGGDGFYAMDYWGQGTLVTVSS

SEQ ID NO: 27 - protein, 119 aa, Artificial Sequence
  source: /note="Description of Artificial Sequence: Synthetic polypeptide"
EVQLVESGGGLVQPGGSLRLSCAASGFNIKDTYIHWVRQAPGKGLEWVARIYPTNAYTRYADSVKGRFTISADTSKNTAYLQMNSLRAEDTAVYYCSRWGGTGFYAMDYWGQGTLVTVS

SEQ ID NO: 28 - protein, 119 aa, Artificial Sequence
  source: /note="Description of Artificial Sequence: Synthetic polypeptide"
EVQLVESGGGLVQPGGSLRLSCAASGFNIKDTYIHWVRQAPGKGLEWVARIYPTEGYTRYADSVKGRFTISADTSKNTAYLQMNSLRAEDTAVYYCSRWGGDSFYAMDYWGQGTLVTVS

SEQ ID NO: 29 - protein, 119 aa, Artificial Sequence
  source: /note="Description of Artificial Sequence: Synthetic polypeptide"
EVQLVESGGGLVQPGGSLRLSCAASGFNIKDTYIHWVRQAPGKGLEWVARIYPTAGYTRYADSVKGRFTISADTSKNTAYLQMNSLRAEDTAVYYCSRWGGDSFYAMDYWGQGTLVTVS

SEQ ID NO: 30 - protein, 119 aa, Artificial Sequence
  source: /note="Description of Artificial Sequence: Synthetic polypeptide"
EVQLVESGGGLVQPGGSLRLSCAASGFNIKDTYIHWVRQAPGKGLEWVARIYPTNGYTRYADSVKGRFTISADTSKNTAYLQMNSLRAEDTAVYYCSRWGGEGFYAMDYWGQGTLVTVS

SEQ ID NO: 31 - protein, 107 aa, Artificial Sequence; identical to SEQ ID NO: 6
  source: /note="Description of Artificial Sequence: Synthetic polypeptide"

SEQ ID NO: 32 - protein, 119 aa, Artificial Sequence
  source: /note="Description of Artificial Sequence: Synthetic polypeptide"
EVQLVESGGGLVQPGGSLRLSCAASGFNIKDTYIHWVRQAPGKGLEWVARIYPTEGYTRYADSVKGRFTISADTSKNTAYLQMNSLRAEDTAVYYCSRWGGDGFYAMDYWGQGTLVTVS

SEQ ID NO: 33 - protein, 107 aa, Artificial Sequence
  source: /note="Description of Artificial Sequence: Synthetic polypeptide"
DIQMTQSPSSLSASVGDRVTITCRASQDVNDAVAWYQQKPGKAPKLLIYSASFLYSGVPSRFSGSRSGTDFTLTISSLQPEDFATYYCQQHYTTPPTFGQGTKVEIK

SEQ ID NO: 34 - protein, 119 aa, Artificial Sequence
  source: /note="Description of Artificial Sequence: Synthetic polypeptide"
EVQLVESGGGLVQPGGSLRLSCAASGFNIKDTYIHWVRQAPGKGLEWVARIYPTNAYTRYADSVKGRFTISADTSKNTAYLQMNSLRAEDTAVYYCSRWGGEGFYAMDYWGQGTLVTVS

SEQ ID NO: 35 - protein, 119 aa, Artificial Sequence; identical to SEQ ID NO: 30
  source: /note="Description of Artificial Sequence: Synthetic polypeptide"

SEQ ID NO: 36 - protein, 107 aa, Artificial Sequence; identical to SEQ ID NO: 33
  source: /note="Description of Artificial Sequence: Synthetic polypeptide"

SEQ ID NO: 37 - protein, 119 aa, Artificial Sequence; identical to SEQ ID NO: 30
  source: /note="Description of Artificial Sequence: Synthetic polypeptide"

SEQ ID NO: 38 - protein, 107 aa, Artificial Sequence
  source: /note="Description of Artificial Sequence: Synthetic polypeptide"
DIQMTQSPSSLSASVGDRVTITCRASQDVQTAVAWYQQKPGKAPKLLIYSASFLYSGVPSRFSGSRSGTDFTLTISSLQPEDFATYYCQQHYTTPPTFGQGTKVEIK

SEQ ID NO: 39 - protein, 119 aa, Artificial Sequence
  source: /note="Description of Artificial Sequence: Synthetic polypeptide"
EVQLVESGGGLVQPGGSLRLSCAASGFNIKDTYIHWVRQAPGKGLEWVARIYPTSGYTRYADSVKGRFTISADTSKNTAYLQMNSLRAEDTAVYYCSRWGGSGFYAMDYWGQGTLVTVS

SEQ ID NO: 40 - protein, 119 aa, Artificial Sequence
  source: /note="Description of Artificial Sequence: Synthetic polypeptide"
EVQLVESGGGLVQPGGSLRLSCAASGFNIKDTYIHWVRQAPGKGLEWVARIYPTAGYTRYADSVKGRFTISADTSKNTAYLQMNSLRAEDTAVYYCSRWGGDGFYAMDYWGQGTLVTVS

SEQ ID NO: 41 - protein, 107 aa, Artificial Sequence; identical to SEQ ID NO: 14
  source: /note="Description of Artificial Sequence: Synthetic polypeptide"

SEQ ID NO: 42 - protein, 107 aa, Artificial Sequence; identical to SEQ ID NO: 14
  source: /note="Description of Artificial Sequence: Synthetic polypeptide"

SEQ ID NO: 43 - protein, 119 aa, Artificial Sequence
  source: /note="Description of Artificial Sequence: Synthetic polypeptide"
EVQLVESGGGLVQPGGSLRLSCAASGFNIKDTYIHWVRQAPGKGLEWVARIYPTSGYTRYADSVKGRFTISADTSKNTAYLQMNSLRAEDTAVYYCSRWGGDTFYAMDYWGQGTLVTVS

SEQ ID NO: 44 - protein, 107 aa, Artificial Sequence
  source: /note="Description of Artificial Sequence: Synthetic polypeptide"
DIQMTQSPSSLSASVGDRVTITCRASQDVETAVAWYQQKPGKAPKLLIYSASFLYSGVPSRFSGSRSGTDFTLTISSLQPEDFATYYCQQHYTTPPTFGQGTKVEIK

SEQ ID NO: 45 - protein, 119 aa, Artificial Sequence
  source: /note="Description of Artificial Sequence: Synthetic polypeptide"
EVQLVESGGGLVQPGGSLRLSCAASGFNIKDTYIHWVRQAPGKGLEWVARIYPTSGYTRYADSVKGRFTISADTSKNTAYLQMNSLRAEDTAVYYCSRWGGDGFYAMDYWGQGTLVTVS

SEQ ID NO: 46 - protein, 119 aa, Artificial Sequence
  source: /note="Description of Artificial Sequence: Synthetic polypeptide"
EVQLVESGGGLVQPGGSLRLSCAASGFNIKDTYIHWVRQAPGKGLEWVARIYPTAGYTRYADSVKGRFTISADTSKNTAYLQMNSLRAEDTAVYYCSRWGGDTFYAMDYWGQGTLVTVS

SEQ ID NO: 47 - protein, 11 aa, Artificial Sequence
  source: /note="Description of Artificial Sequence: Synthetic peptide"
RASQDVNTAVA

SEQ ID NO: 48 - protein, 7 aa, Artificial Sequence
  source: /note="Description of Artificial Sequence: Synthetic peptide"
SASFLYS

SEQ ID NO: 49 - protein, 9 aa, Artificial Sequence
  source: /note="Description of Artificial Sequence: Synthetic peptide"
QQHYTTPPT

SEQ ID NO: 50 - protein, 5 aa, Artificial Sequence
  source: /note="Description of Artificial Sequence: Synthetic peptide"
DTYIH

SEQ ID NO: 51 - protein, 17 aa, Artificial Sequence
  source: /note="Description of Artificial Sequence: Synthetic peptide"
RIYPTNGYTRYADSVKG

SEQ ID NO: 52 - protein, 11 aa, Artificial Sequence
  source: /note="Description of Artificial Sequence: Synthetic peptide"
WGGDGFYAMDY

SEQ ID NO: 53 - protein, 11 aa, Artificial Sequence
  source: /note="Description of Artificial Sequence: Synthetic peptide"
RASQDVDTAVA

SEQ ID NO: 54 - protein, 11 aa, Artificial Sequence
  source: /note="Description of Artificial Sequence: Synthetic peptide"
RASQDVSTAVA

SEQ ID NO: 55 - protein, 11 aa, Artificial Sequence
  source: /note="Description of Artificial Sequence: Synthetic peptide"
RASQDVTTAVA

SEQ ID NO: 56 - protein, 11 aa, Artificial Sequence
  source: /note="Description of Artificial Sequence: Synthetic peptide"
RASQDVQTAVA

SEQ ID NO: 57 - protein, 17 aa, Artificial Sequence
  source: /note="Description of Artificial Sequence: Synthetic peptide"
RIYPTEGYTRYADSVKG

SEQ ID NO: 58 - protein, 17 aa, Artificial Sequence
  source: /note="Description of Artificial Sequence: Synthetic peptide"
RIYPTNAYTRYADSVKG

SEQ ID NO: 59 - protein, 17 aa, Artificial Sequence
  source: /note="Description of Artificial Sequence: Synthetic peptide"
RIYPTEGYTRYADSVKG

SEQ ID NO: 60 - protein, 17 aa, Artificial Sequence
  source: /note="Description of Artificial Sequence: Synthetic peptide"
RIYPTAGYTRYADSVKG

SEQ ID NO: 61 - protein, 17 aa, Artificial Sequence
  source: /note="Description of Artificial Sequence: Synthetic peptide"
RIYPTSGYTRYADSVKG

SEQ ID NO: 62 - protein, 11 aa, Artificial Sequence
  source: /note="Description of Artificial Sequence: Synthetic peptide"
WGGDSFYAMDY

SEQ ID NO: 63 - protein, 11 aa, Artificial Sequence
  source: /note="Description of Artificial Sequence: Synthetic peptide"
WGGTGFYAMDY

SEQ ID NO: 64 - protein, 11 aa, Artificial Sequence
  source: /note="Description of Artificial Sequence: Synthetic peptide"
WGGSGFYAMDY

SEQ ID NO: 65 - protein, 12 aa, Artificial Sequence
  source: /note="Description of Artificial Sequence: Synthetic peptide"
RWGGEGFYAMDY

SEQ ID NO: 66 - protein, 5 aa, Artificial Sequence
  source: /note="Description of Artificial Sequence: Synthetic peptide"
NYYIH

SEQ ID NO: 67 - protein, 17 aa, Artificial Sequence
  source: /note="Description of Artificial Sequence: Synthetic peptide"
WIYPGDGNTKYNEKFKG

SEQ ID NO: 68 - protein, 10 aa, Artificial Sequence
  source: /note="Description of Artificial Sequence: Synthetic peptide"
DSYSNYYFDY

SEQ ID NO: 69 - protein, 17 aa, Artificial Sequence
  source: /note="Description of Artificial Sequence: Synthetic peptide"
KSSQSLLNSRTRKNYLA

SEQ ID NO: 70 - protein, 7 aa, Artificial Sequence
  source: /note="Description of Artificial Sequence: Synthetic peptide"
WASTRES

SEQ ID NO: 71 - protein, 8 aa, Artificial Sequence
  source: /note="Description of Artificial Sequence: Synthetic peptide"
TQSFILRT

SEQ ID NO: 72 - protein, 5 aa, Artificial Sequence
  source: /note="Description of Artificial Sequence: Synthetic peptide"
SYYIH

SEQ ID NO: 73 - protein, 17 aa, Artificial Sequence
  source: /note="Description of Artificial Sequence: Synthetic peptide"
WIYPENDNTKYNEKFKD

SEQ ID NO: 74 - protein, 10 aa, Artificial Sequence
  source: /note="Description of Artificial Sequence: Synthetic peptide"
DGYSRYYFDY

SEQ ID NO: 75 - protein, 7 aa, Artificial Sequence
  source: /note="Description of Artificial Sequence: Synthetic peptide"
WTSTRKS

SEQ ID NO: 76 - protein, 8 aa, Artificial Sequence
  source: /note="Description of Artificial Sequence: Synthetic peptide"
KQSFILRT

SEQ ID NO: 77 - protein, 119 aa, Artificial Sequence
  source: /note="Description of Artificial Sequence: Synthetic polypeptide"
EVQLVQSGAEVKKPGASVKVSCKASGYTFTNYYIHWVRQAPGQGLEWIGWIYPGDGNTKYNEKFKGRATLTADTSTSTAYLELSSLRSEDTAVYYCARDSYSNYYFDYWGQGTLVTVSS

SEQ ID NO: 78 - protein, 112 aa, Artificial Sequence
  source: /note="Description of Artificial Sequence: Synthetic polypeptide"
DIVMTQSPDSLAVSLGERATINCKSSQSLLNSRTRKNYLAWYQQKPGQPPKLLIYWASTRESGVPDRFSGSGSGTDFTLTISSLQAEDVAVYYCTQSFILRTFGQGTKVEIK

SEQ ID NO: 79 - protein, 119 aa, Artificial Sequence
  source: /note="Description of Artificial Sequence: Synthetic polypeptide"
EVQLVQSGAEVKKPGASVKVSCKASGFTFTSYYIHWVRQAPGQGLEWIGWIYPENDNTKYNEKFKDRVTITADTSTSTAYLELSSLRSEDTAVYYCARDGYSRYYFDYWGQGTLVTVSS

SEQ ID NO: 80 - protein, 112 aa, Artificial Sequence
  source: /note="Description of Artificial Sequence: Synthetic polypeptide"
DIVMTQSPDSLAVSLGERATINCKSSQSLLNSRTRKNYLAWYQQKPGQSPKLLIYWTSTRKSGVPDRFSGSGSGTDFTLTISSLQAEDVAVYYCKQSFILRTFGQGTKVEIK

SEQ ID NO: 81 - protein, 112 aa, Artificial Sequence
  source: /note="Description of Artificial Sequence: Synthetic polypeptide"
DIVMTQSPDSLAVSLGERATINCKSSQSLLNSRTRKNYLAWYQQKPGQSPKLLIYWTSTRKSGVPDRFSGSGSGTDFTLTISSLQAEDVAVYYCTQSFILRTFGQGTKVEIK

SEQ ID NO: 82 - protein, 27 aa, Artificial Sequence
  source: /note="Description of Artificial Sequence: Synthetic peptide"
QDGNEEMGGITQTPYKVSISGTTVILT

SEQ ID NO: 83 - protein, 28 aa, Artificial Sequence
  source: /note="Description of Artificial Sequence: Synthetic peptide"
QDGNEEMGGITQTPYKVSISGTTVILTC

SEQ ID NO: 84 - protein, 5 aa, Artificial Sequence
  source: /note="Description of Artificial Sequence: Synthetic peptide"
  VARIANT (1)..(1): /replace="Ser"
  MISC_FEATURE (1)..(5): /note="Variant residues given in the sequence have no preference with respect to those in the annotations for variant positions"
NYYIH

SEQ ID NO: 85 - protein, 17 aa, Artificial Sequence
  source: /note="Description of Artificial Sequence: Synthetic peptide"
  VARIANT (5)..(5): /replace="Glu"
  VARIANT (6)..(6): /replace="Asn"
  VARIANT (7)..(7): /replace="Gly"
  VARIANT (17)..(17): /replace="Gly"
  MISC_FEATURE (1)..(17): /note="Variant residue given in the sequence has no preference with respect to that in the annotations for variant position"
WIYPGDDNTKYNEKFKD

SEQ ID NO: 86 - protein, 10 aa, Artificial Sequence
  source: /note="Description of Artificial Sequence: Synthetic peptide"
  VARIANT (2)..(2): /replace="Gly"
  VARIANT (5)..(5): /replace="Arg"
  MISC_FEATURE (1)..(10): /note="Variant residue given in the sequence has no preference with respect to that in the annotations for variant position"
DSYSNYYFDY

SEQ ID NO: 87 - protein, 7 aa, Artificial Sequence
  source: /note="Description of Artificial Sequence: Synthetic peptide"
  VARIANT (2)..(2): /replace="Thr"
  VARIANT (6)..(6): /replace="Lys"
  MISC_FEATURE (1)..(7): /note="Variant residue given in the sequence has no preference with respect to that in the annotations for variant position"
WASTRES

SEQ ID NO: 88 - protein, 8 aa, Artificial Sequence
  source: /note="Description of Artificial Sequence: Synthetic peptide"
  VARIANT (1)..(1): /replace="Thr"
  MISC_FEATURE (1)..(8): /note="Variant residue given in the sequence has no preference with respect to that in the annotations for variant position"
KQSFILRT

SEQ ID NO: 89 - protein, 16 aa, Homo sapiens
QDGNEEMGGITQTPYK